European Patent Application EP 4 190 914 A1, published June 7, 2023. Title: Major Histocompatibility Complex Single Nucleotide Polymorphisms. Applicant: Illumina, Inc. Application EP. The sequence listing filed with the application follows.

SEQUENCE LISTING (50 sequences)

SEQ ID NO: 1 - protein, 6 aa, Homo sapiens
PCPVLD

SEQ ID NO: 2 - protein, 6 aa, Homo sapiens
LSPVIH

SEQ ID NO: 3 - DNA, 19 bp, synthetic construct
  misc_feature 1..19: note = C4A control forward primer
  source 1..19: mol_type = other DNA
gacccctgtccagtgttag

SEQ ID NO: 4 - DNA, 20 bp, synthetic construct
  misc_feature 1..20: note = C4A control reverse primer
  source 1..20: mol_type = other DNA
cctcctctgagtcttcatcc

SEQ ID NO: 5 - DNA, 23 bp, synthetic construct
  misc_feature 1..23: note = T9763 forward primer
  source 1..23: mol_type = other DNA
ccccgggtttctgtctatagagt

SEQ ID NO: 6 - DNA, 20 bp, synthetic construct
  misc_feature 1..20: note = T9763 reverse primer
  source 1..20: mol_type = other DNA
tgccaggtgatggtccacaa

SEQ ID NO: 7 - DNA, 19 bp, synthetic construct
  misc_feature 1..19: note = C9796 forward primer
  source 1..19: mol_type = other DNA
tcctcgtgttggggacacc

SEQ ID NO: 8 - DNA, 21 bp, synthetic construct
  misc_feature 1..21: note = C9796 reverse primer
  source 1..21: mol_type = other DNA
agagtggttgcctcttcatgg

SEQ ID NO: 9 - DNA, 24 bp, synthetic construct
  misc_feature 1..24: note = T9881 forward primer
  source 1..24: mol_type = other DNA
caggacattcagcaaaacaccgat

SEQ ID NO: 10 - DNA, 20 bp, synthetic construct
  misc_feature 1..20: note = T9881 reverse primer
  source 1..20: mol_type = other DNA
gcctggctatcgctggatgt

SEQ ID NO: 11 - DNA, 21 bp, synthetic construct
  misc_feature 1..21: note = T10289 forward primer
  source 1..21: mol_type = other DNA
ccaactccctgcgagtggatg

SEQ ID NO: 12 - DNA, 18 bp, synthetic construct
  misc_feature 1..18: note = T10289 reverse primer
  source 1..18: mol_type = other DNA
ctccagctggcaggggca

SEQ ID NO: 13 - DNA, 20 bp, synthetic construct
  misc_feature 1..20: note = T10309 forward primer
  source 1..20: mol_type = other DNA
ctctcccactctgacctcct

SEQ ID NO: 14 - DNA, 21 bp, synthetic construct
  misc_feature 1..21: note = T10309 reverse primer
  source 1..21: mol_type = other DNA
ggaacacctgaagggcactgt

SEQ ID NO: 15 - DNA, 20 bp, synthetic construct
  misc_feature 1..20: note = C10676 forward primer
  source 1..20: mol_type = other DNA
acatgtcccacgtcctctcc

SEQ ID NO: 16 - DNA, 19 bp, synthetic construct
  misc_feature 1..19: note = C10676 reverse primer
  source 1..19: mol_type = other DNA
atccttggctggaagctcg

SEQ ID NO: 17 - DNA, 20 bp, synthetic construct
  misc_feature 1..20: note = A11437 forward primer
  source 1..20: mol_type = other DNA
gacacgtctgcccatgatga

SEQ ID NO: 18 - DNA, 20 bp, synthetic construct
  misc_feature 1..20: note = A11437 reverse primer
  source 1..20: mol_type = other DNA
ggcccagacagggtgacatc

SEQ ID NO: 19 - DNA, 17 bp, synthetic construct
  misc_feature 1..17: note = A11483 forward primer
  source 1..17: mol_type = other DNA
cagcagccggactgcca

SEQ ID NO: 20 - DNA, 22 bp, synthetic construct
  misc_feature 1..22: note = A11483 reverse primer
  source 1..22: mol_type = other DNA
aggtcctcctcctgcaggatct

SEQ ID NO: 21 - DNA, 20 bp, synthetic construct
  misc_feature 1..20: note = G12071 forward primer
  source 1..20: mol_type = other DNA
cactgtggctccccgactct

SEQ ID NO: 22 - DNA, 20 bp, synthetic construct
  misc_feature 1..20: note = G12071 reverse primer
  source 1..20: mol_type = other DNA
tcagtctgcctctgccctcc

SEQ ID NO: 23 - DNA, 20 bp, synthetic construct
  misc_feature 1..20: note = A12152 forward primer
  source 1..20: mol_type = other DNA
tgggcacagtggcagagatt

SEQ ID NO: 24 - DNA, 20 bp, synthetic construct
  misc_feature 1..20: note = A12512 reverse primer
  source 1..20: mol_type = other DNA
tgtctgggcctcaggtgacc

SEQ ID NO: 25 - DNA, 15 bp, synthetic construct
  misc_feature 1..15: note = A12568 - A12837 forward primer
  source 1..15: mol_type = other DNA
tgcccacggaagcca

SEQ ID NO: 26 - DNA, 21 bp, synthetic construct
  misc_feature 1..21: note = A12568 - A12837 reverse primer
  source 1..21: mol_type = other DNA
ctacagcctgcccttctagca

SEQ ID NO: 27 - DNA, 20 bp, synthetic construct
  misc_feature 1..20: note = G12479 forward primer
  source 1..20: mol_type = other DNA
ggccaggtgcccaacagccg

SEQ ID NO: 28 - DNA, 20 bp, synthetic construct
  misc_feature 1..20: note = G12749 reverse primer
  source 1..20: mol_type = other DNA
ggccaggtgcccaacagccg

SEQ ID NO: 29 - DNA, 21 bp, synthetic construct
  misc_feature 1..21: note = A13189 forward primer
  source 1..21: mol_type = other DNA
gccaccttcggattgatgtga

SEQ ID NO: 30 - DNA, 20 bp, synthetic construct
  misc_feature 1..20: note = A13189 reverse primer
  source 1..20: mol_type = other DNA
cagcctcgaggaagcctcaa

SEQ ID NO: 31 - DNA, 20 bp, synthetic construct
  misc_feature 1..20: note = C13193 forward primer
  source 1..20: mol_type = other DNA
cttcggattcatgtgggacc

SEQ ID NO: 32 - DNA, 20 bp, synthetic construct
  misc_feature 1..20: note = C13193 reverse primer
  source 1..20: mol_type = other DNA
cttggtctcgggaggcagtg

SEQ ID NO: 33 - DNA, 20 bp, synthetic construct
  misc_feature 1..20: note = T14563 forward primer
  source 1..20: mol_type = other DNA
ggtgaggggtgaggggctct

SEQ ID NO: 34 - DNA, 20 bp, synthetic construct
  misc_feature 1..20: note = T14563 reverse primer
  source 1..20: mol_type = other DNA
cccttggtctgaggactacc

SEQ ID NO: 35 - DNA, 20 bp, synthetic construct
  misc_feature 1..20: note = T14757 forward primer
  source 1..20: mol_type = other DNA
ccctgccttcctgtttactt

SEQ ID NO: 36 - DNA, 20 bp, synthetic construct
  misc_feature 1..20: note = T14757 reverse primer
  source 1..20: mol_type = other DNA
cccttggtctgaggactacc

SEQ ID NO: 37 - DNA, 20 bp, synthetic construct
  misc_feature 1..20: note = A14831 forward primer
  source 1..20: mol_type = other DNA
atgccgtgtcgcccatccca

SEQ ID NO: 38 - DNA, 20 bp, synthetic construct
  misc_feature 1..20: note = A14831 reverse primer
  source 1..20: mol_type = other DNA
cccttggtctgaggactacc

SEQ ID NO: 39 - DNA, 20 bp, synthetic construct
  misc_feature 1..20: note = T14592 forward primer
  source 1..20: mol_type = other DNA
agagatggcagaccaggctt

SEQ ID NO: 40 - DNA, 20 bp, synthetic construct
  misc_feature 1..20: note = T14952 reverse primer
  source 1..20: mol_type = other DNA
agtggttcaccagggagtgg

SEQ ID NO: 41 - DNA, 21 bp, synthetic construct
  misc_feature 1..21: note = G15108 forward primer
  source 1..21: mol_type = other DNA
tgccctgtctgcctactggat

SEQ ID NO: 42 - DNA, 18 bp, synthetic construct
  misc_feature 1..18: note = G15108 reverse primer
  source 1..18: mol_type = other DNA
ctcaaaacagccgcaccc

SEQ ID NO: 43 - DNA, 20 bp, synthetic construct
  misc_feature 1..20: note = C16954 forward primer
  source 1..20: mol_type = other DNA
acatgtcccacgtcctctcc

SEQ ID NO: 44 - DNA, 25 bp, synthetic construct
  misc_feature 1..25: note = C16954 reverse primer
  source 1..25: mol_type = other DNA
catagtcctcatagtcctcgtttgg

SEQ ID NO: 45 - DNA, 20 bp, synthetic construct
  misc_feature 1..20: note = T17316 forward primer
  source 1..20: mol_type = other DNA
ccagccaaggatgacccaga

SEQ ID NO: 46 - DNA, 17 bp, synthetic construct
  misc_feature 1..17: note = T17316 reverse primer
  source 1..17: mol_type = other DNA
ggtcagcacgcagggca

SEQ ID NO: 47 - DNA, 20 bp, synthetic construct
  misc_feature 1..20: note = T19588 forward primer
  source 1..20: mol_type = other DNA
ccctccctcggggaccggct

SEQ ID NO: 48 - DNA, 21 bp, synthetic construct
  misc_feature 1..21: note = T19588 reverse primer
  source 1..21: mol_type = other DNA
tcacacttccagatggtcagg

SEQ ID NO: 49 - DNA, 21 bp, synthetic construct
  misc_feature 1..21: note = A20170 forward primer
  source 1..21: mol_type = other DNA
tttgctctgacaccaacttcc

SEQ ID NO: 50 - DNA, 20 bp, synthetic construct
  misc_feature 1..20: note = A20170 reverse primer
  source 1..20: mol_type = other DNA
ggtcataggtggccgcatct